European Patent Application EP 4 148 143 A1, published March 15, 2023. Title: POLYPURINE REVERSE HOOGSTEEN HAIRPINS AND PARALLEL CLAMPS AND THEIR USE AS BIOSENSORS. Applicant: Consejo Superior de Investigaciones Científicas Universitat Barcelona CONSORCIO CENTRO DE INVESTIGACIÓN BIOMÉDICA EN RED, M.P. The sequence listing filed with the application follows.

SEQUENCE LISTING (80 sequences)

SEQ ID NO: 1 - DNA, 51 bp, Artificial Sequence
  CC1PPRH-amino
tttttgagcagaagggtagtagagagttttgagagatgatgggaagacgag

SEQ ID NO: 2 - DNA, 46 bp, Artificial Sequence
  CC1PPRH (gel assays)
gagcagaagggtagtagagagttttgagagatgatgggaagacgag

SEQ ID NO: 3 - DNA, 26 bp, Artificial Sequence
  CC1duplex-amino
tttttgagcagaagggtagtagagag

SEQ ID NO: 4 - DNA, 51 bp, Artificial Sequence
  AA1ParallelClamp-amino
  misc_feature 1..26: /note="Sequence in the 5' to 3' direction"
  misc_feature 27..30: /note="linker"
  misc_feature 31-51: /note="Sequence in the 3' to 5' direction"
tttttgagcagaagggtagtagagagttttctctctgctgcccttctcctc

SEQ ID NO: 5 - DNA, 20 bp, Artificial Sequence
  CC1 second oligonucleotide
ggccaatagcaaaatgactc

SEQ ID NO: 6 - DNA, 44 bp, Artificial Sequence
  CC1target
gagtcattttgctattggcctagctctctactacccttctgctc

SEQ ID NO: 7 - DNA, 47 bp, Artificial Sequence
  CC1-FAMtarget
gctattggcctagctctctactacccttctgctcgcatagtgtatac

SEQ ID NO: 8 - RNA, 30 nt, Artificial Sequence
  CC1RNAtarget-FAM
cuagcucucuacuacccuucugcucgcaua

SEQ ID NO: 9 - DNA, 51 bp, Artificial Sequence
  CC2PPRH-amino
tttttgtgatgaggaacgagaagaggttttggagaagagcaaggagtagtg

SEQ ID NO: 10 - DNA, 46 bp, Artificial Sequence
  CC2PPRH (gel assays)
gtgatgaggaacgagaagaggttttggagaagagcaaggagtagtg

SEQ ID NO: 11 - DNA, 26 bp, Artificial Sequence
  CC2duplex-amino
tttttgtgatgaggaacgagaagagg

SEQ ID NO: 12 - DNA, 19 bp, Artificial Sequence
  CC2-biotineRP
tgcgtagaagccttttggc

SEQ ID NO: 13 - DNA, 20 bp, Artificial Sequence
  CC2-biotineRPNew
ccttctgcgtagaagccttt

SEQ ID NO: 14 - DNA, 65 bp, Artificial Sequence
  CC2DNATarget
gccaaaaggcttctacgcagaagggagcagaggcggcagtcaagcctcttctcgttcctcatcac

SEQ ID NO: 15 - DNA, 61 bp, Artificial Sequence
  CC2NewTarget
aaaggcttctacgcagaagggagcagaggcggcagtcaagcctcttctcgttcctcatcac

SEQ ID NO: 16 - DNA, 49 bp, Artificial Sequence
  CC3PPRH-amino
tttttgagggaaggacataagatgattttagtagaatacaggaagggag

SEQ ID NO: 17 - DNA, 44 bp, Artificial Sequence
  CC3PPRH (gel assay)
gagggaaggacataagatgattttagtagaatacaggaagggag

SEQ ID NO: 18 - DNA, 25 bp, Artificial Sequence
  CC3duplex-amino
tttttgagggaaggacataagatga

SEQ ID NO: 19 - DNA, 20 bp, Artificial Sequence
  CC3-second oligonucleotide
ccctttccacaaaaatcaac

SEQ ID NO: 20 - DNA, 43 bp, Artificial Sequence
  CC3target
gttgatttttgtggaaagggctatcatcttatgtccttccctc

SEQ ID NO: 21 - DNA, 47 bp, Artificial Sequence
  CC3-FAMtarget
gtggaaagggctatcatcttatgtccttccctcagtcagcacctcat

SEQ ID NO: 22 - RNA, 30 nt, Artificial Sequence
  CC3RNAtarget
ggcuaucaucuuauguccuucccucaguca

SEQ ID NO: 23 - DNA, 44 bp, Artificial Sequence
  HRSV1PPRHamino
aaaagagatgggagaagtggttttggtgaagagggtagagaaaa

SEQ ID NO: 24 - DNA, 44 bp, Artificial Sequence
  HRSV2PPRHamino
agggtaacaaaggaaaggtattttatggaaaggaaacaatggga

SEQ ID NO: 25 - DNA, 20 bp, Artificial Sequence
  HRSV1RPbiotin
cagaatataggcatgactct

SEQ ID NO: 26 - DNA, 20 bp, Artificial Sequence
  HRSV2RPbiotin
agcttttaatatttgcatcg

SEQ ID NO: 27 - DNA, 43 bp, Artificial Sequence
  HRSV1DNAtarget
agagtcatgcctatattctggagccacttctcccatctctttt

SEQ ID NO: 28 - DNA, 43 bp, Artificial Sequence
  HRSV2target
cgatgcaaatattaaaagcttaatacctttcctttgttaccct

SEQ ID NO: 29 - DNA, 30 bp, Artificial Sequence
  HRSV1FAMTarget
tggagccacttctcccatctcttttagcat

SEQ ID NO: 30 - DNA, 30 bp, Artificial Sequence
  HRSV2FAMTarget
cttaatacctttcctttgttaccctataac

SEQ ID NO: 31 - DNA, 59 bp, Artificial Sequence
  CCIZ2-PPRH-amino
tttttagagaaagagacgggtgagagacaattttaacagagagtgggcagagaaagaga

SEQ ID NO: 32 - DNA, 53 bp, Artificial Sequence
  CCIZ8-PPRH-amino
tttttggaagagaaggcaatggtgaaattttaaagtggtaacggaagagaagg

SEQ ID NO: 33 - DNA, 20 bp, Artificial Sequence
  CCIZ2-RP-biotine
gactaagaaaatgataacac

SEQ ID NO: 34 - DNA, 20 bp, Artificial Sequence
  CCIZ8-RP-biotine
cgccaacaattgctccctct

SEQ ID NO: 35 - DNA, 48 bp, Artificial Sequence
  CCIZ2-DNAtarget
gtgttatcattttcttagtcatattgtctctcacccgtctctttctct

SEQ ID NO: 36 - DNA, 45 bp, Artificial Sequence
  CCIZ8-DNA Target
agagggagcaattgttggcgaaatttcaccattgccttctcttcc

SEQ ID NO: 37 - DNA, 30 bp, Artificial Sequence
  H1N1-PB1target-FAM
tattgtctctcacccgtctctttctctgaa

SEQ ID NO: 38 - DNA, 30 bp, Artificial Sequence
  H1N1-NEPtarget-FAM
gaaatttcaccattgccttctcttccagga

SEQ ID NO: 39 - DNA, 21 bp, Artificial Sequence
  Sequence from the Example
gagcagaagggtagtagagag

SEQ ID NO: 40 - DNA, 21 bp, Artificial Sequence
  Sequence from the Examples
ctctctactacccttctgctc

SEQ ID NO: 41 - DNA, 21 bp, Artificial Sequence
  Sequence from the Examples
gtgatgaggaacgagaagagg

SEQ ID NO: 42 - DNA, 21 bp, Artificial Sequence
  Sequence from the Examples
cctcttctcgttcctcatcac

SEQ ID NO: 43 - DNA, 20 bp, Artificial Sequence
  Sequence from the Examples
gagggaaggacataagatga

SEQ ID NO: 44 - DNA, 20 bp, Artificial Sequence
  Sequence from the Examples
tcatcttatgtccttccctc

SEQ ID NO: 45 - DNA, 21 bp, Artificial Sequence
  Sequence from the Examples
ctctctattacccatctgctc

SEQ ID NO: 46 - skipped

SEQ ID NO: 47 - DNA, 14 bp, Artificial Sequence
  Sequence from the Examples
cttatgtccttccc

SEQ ID NO: 48-49 - skipped (2 entries)

SEQ ID NO: 50 - DNA, 10 bp, Artificial Sequence
  Sequence from the Examples
catcttatgt

SEQ ID NO: 51 - DNA, 43 bp, Artificial Sequence
  Sequence from the Examples
aaaagagatgggagaagtggctccagaatataggcatgactct

SEQ ID NO: 52 - DNA, 20 bp, Artificial Sequence
  Sequence from the Examples
agggtaacaaaggaaaggta

SEQ ID NO: 53 - DNA, 20 bp, Artificial Sequence
  Sequence from the Examples
tacctttcctttgttaccct

SEQ ID NO: 54 - DNA, 20 bp, Artificial Sequence
  Sequence from the Examples
cgatgcaaatattaaaagct

SEQ ID NO: 55 - skipped

SEQ ID NO: 56 - DNA, 25 bp, Artificial Sequence
  Sequence from the Examples
tatgactaagaaaatgataacacag

SEQ ID NO: 57 - DNA, 25 bp, Artificial Sequence
  Sequence from the Examples
ctgtgttatcattttcttagtcata

SEQ ID NO: 58 - DNA, 20 bp, Artificial Sequence
  Sequence from the Examples
gtgttatcattttcttagtc

SEQ ID NO: 59 - DNA, 48 bp, Artificial Sequence
  CCIZ8-PPRH (gel assay)
ggaagagaaggcaatggtgaaattttaaagtggtaacggaagagaagg

SEQ ID NO: 60 - DNA, 43 bp, Artificial Sequence
  CC1PPRH
  misc_feature 22: /note="N= linker molecule"
gagcagaagggtagtagagagngagagatgatgggaagacgag

SEQ ID NO: 61 - DNA, 46 bp, Artificial Sequence
  AA1ParallelClamp
  misc_feature 1..21: /note="Sequence in the 5' to 3' direction"
  misc_feature 22..25: /note="linker"
  misc_feature 26-46: /note="Sequence in the 3' to 5' direction"
gagcagaagggtagtagagagttttctctctgctgcccttctcctc

SEQ ID NO: 62 - DNA, 43 bp, Artificial Sequence
  AA1ParallelClamp
  misc_feature 1..21: /note="Sequence in the 5' to 3' direction"
  misc_feature 22: /note="N= Linker molecule"
  misc_feature 23..43: /note="From nucleotide 23 to 46 the direction is 3'-5'"
gagcagaagggtagtagagagnctctctgctgcccttctcctc

SEQ ID NO: 63 - DNA, 43 bp, Artificial Sequence
  CC2PPRH
  misc_feature 22: /note="N= linker molecule"
gtgatgaggaacgagaagaggnggagaagagcaaggagtagtg

SEQ ID NO: 64 - DNA, 41 bp, Artificial Sequence
  CC3PPRH
  misc_feature 21: /note="N= linker molecule"
gagggaaggacataagatganagtagaatacaggaagggag

SEQ ID NO: 65 - DNA, 41 bp, Artificial Sequence
  HRSV1PPRH
  misc_feature 21: /note="N= linker molecule"
aaaagagatgggagaagtggnggtgaagagggtagagaaaa

SEQ ID NO: 66 - DNA, 41 bp, Artificial Sequence
  HRSV2PPR
  misc_feature 21: /note="N=Linker molecule"
agggtaacaaaggaaaggtanatggaaaggaaacaatggga

SEQ ID NO: 67 - DNA, 51 bp, Artificial Sequence
  CCIZ2-PPRH
  misc_feature 26: /note="N= Linker Molecule"
agagaaagagacgggtgagagacaanaacagagagtgggcagagaaagaga

SEQ ID NO: 68 - DNA, 45 bp, Artificial Sequence
  CCIZ8-PPRH
  misc_feature 23: /note="N= linker feature"
ggaagagaaggcaatggtgaaanaaagtggtaacggaagagaagg

SEQ ID NO: 69 - DNA, 20 bp, Artificial Sequence
  Sequence from the Examples
agagggagcaattgttggcg

SEQ ID NO: 70 - DNA, 24 bp, Artificial Sequence
  Seq 1 Table 1
agatgaggatgaagaagaaggtga

SEQ ID NO: 71 - DNA, 20 bp, Artificial Sequence
  Sequence 2 in Table 8
aaaagagatgggagaagtgg

SEQ ID NO: 72 - DNA, 20 bp, Artificial Sequence
  Sequence 2 in Table 8
aaagggaaatggggcaaata

SEQ ID NO: 73 - DNA, 20 bp, Artificial Sequence
  Sequence 3 in Table 8
agcaagaagaggaaacgaag

SEQ ID NO: 74 - DNA, 20 bp, Artificial Sequence
  Sequence 4 in Table 8
agcaagaagaggaaacgaag

SEQ ID NO: 75 - DNA, 20 bp, Artificial Sequence
  Sequence 5 in table 8
agaaaagtatggagatgaag

SEQ ID NO: 76 - DNA, 25 bp, Artificial Sequence
  Sequence 1 in Table 9
agagaaagagacgggtgagagacaa

SEQ ID NO: 77 - DNA, 19 bp, Artificial Sequence
  Sequence 2 in Table 9
agggatgcaaataaggggg

SEQ ID NO: 78 - DNA, 22 bp, Artificial Sequence
  Sequence 1 in table 10
ggaagagaaggcaatggtgaaa

SEQ ID NO: 79 - DNA, 20 bp, Artificial Sequence
  Sequence 2 in Table 10
agaaacgagaaatggcggga

SEQ ID NO: 80 - DNA, 20 bp, Artificial Sequence
  Sequence 3 in Table 10
gaagtggagcaagagataag